European Patent Application EP 4 206 227 A1, published July 5, 2023. Title: ANTI-OX40 ANTIBODY, AND PHARMACEUTICAL COMPOSITION AND APPLICATION THEREOF. Applicant: SHANGHAI ACEMAB CORPORATION LTD. ZHONGSHAN HENGDONG BIOPHARMACEUTICAL CO., LTD. The sequence listing filed with the application follows.

SEQUENCE LISTING (347 sequences)

SEQ ID NO: 1 - protein, 10 aa, Artificial Sequence
  HCDR1
  MUTAGEN (1)..(1): Xaa is G or S
  MUTAGEN (2)..(2): Xaa is A, D, F, G, V or Y
  MUTAGEN (3)..(3): Xaa is S, T or I
  MUTAGEN (4)..(4): Xaa is I, L or F
  MUTAGEN (5)..(5): Xaa is I, S, D, N, T or A
  MUTAGEN (6)..(6): Xaa is N, S, T, D, R or G
  MUTAGEN (7)..(7): Xaa is N, S, T, Y, A, G or F
  MUTAGEN (8)..(8): Xaa is N, Y, A, G, W, S, I, K, F, T or D
  MUTAGEN (9)..(9): Xaa is W, V or null
  MUTAGEN (10)..(10): Xaa is N, G or null
XXXXXXXXXX

SEQ ID NO: 2 - protein, 10 aa, Artificial Sequence
  HCDR2
  MUTAGEN (1)..(1): Xaa is M or I
  MUTAGEN (2)..(2): Xaa is N, Y, S, K, H or F
  MUTAGEN (3)..(3): Xaa is P, W, Q, H, S, G, A or R
  MUTAGEN (4)..(4): Xaa is N, S, G, Y, K or D
  MUTAGEN (5)..(5): Xaa is S, D, G, N, A or T
  MUTAGEN (6)..(6): Xaa is T, N, S, D or G
  MUTAGEN (7)..(7): Xaa is N, K, T, S, D, Y, H, G, A or E
  MUTAGEN (8)..(8): Xaa is T, I, K, G or null
  MUTAGEN (9)..(9): Xaa is T or null
  MUTAGEN (10)..(10): Xaa is T, I or null
XXXXXXXXXX

SEQ ID NO: 3 - protein, 19 aa, Artificial Sequence
  HCDR3
  MUTAGEN (1)..(1): Xaa is V, T, S or A
  MUTAGEN (2)..(2): Xaa is R, K, I, G, A, T, S, H, Q, N or E
  MUTAGEN (3)..(3): Xaa is S, D, W, G, Y, A, E, R, L, V, T, M or K
  MUTAGEN (4)..(4): Xaa is G, Y, F, V, L, A, P, D, S, W, R, Q, E, N or K
  MUTAGEN (5)..(5): Xaa is D, Y, G, S, R, F, T, V, A, P, L, I, E, W or N
  MUTAGEN (6)..(6): Xaa is W, G, E, D, S, R, P, Y, N, L, A, T, I or V
  MUTAGEN (7)..(7): Xaa is H, S, L, A, T, Y, G, F, W, V, E, D or M
  MUTAGEN (8)..(8): Xaa is C, G, L, F, Y, S, W, D, M, T, N, R, H, V or P
  MUTAGEN (9)..(9): Xaa is F, S, D, Y, W, G, T, E, P, L, R, N or null
  MUTAGEN (10)..(10): Xaa is D, Y, F, I, N, W, V, P, E, L, G, S, Q or null
  MUTAGEN (11)..(11): Xaa is Y, G, D, W, F, A, I, Q, S, N or null
  MUTAGEN (12)..(12): Xaa is W, D, Y, F, N, G, R, P or null
  MUTAGEN (13)..(13): Xaa is I, W, Y, D, S, F, G, L or null
  MUTAGEN (14)..(14): Xaa is Q, W, I, Y, F, D, V, H or null
  MUTAGEN (15)..(15): Xaa is H, W, M, D, Y, F or null
  MUTAGEN (16)..(16): Xaa is W, D, S, Y or null
  MUTAGEN (17)..(17): Xaa is V, W, Y or null
  MUTAGEN (18)..(18): Xaa is W or null
  misc_feature (19)..(19): Xaa can be any naturally occurring amino acid
CXXXXXXXXXXXXXXXXXX

SEQ ID NO: 4 - protein, 12 aa, Artificial Sequence
  LCDR1
  MUTAGEN (1)..(1): Xaa is H or Q
  MUTAGEN (2)..(2): Xaa is G, D, S or T
  MUTAGEN (3)..(3): Xaa is S, I, L, T or V
  MUTAGEN (4)..(4): Xaa is S, N, R, W, L, V or F
  MUTAGEN (5)..(5): Xaa is T, D, N, S, H, Y or G
  MUTAGEN (6)..(6): Xaa is Y, D, W, S, R, N, G or T
  MUTAGEN (7)..(7): Xaa is N, D, S, Y or null
  MUTAGEN (8)..(8): Xaa is G, N or null
  MUTAGEN (9)..(9): Xaa is Y, N, D, H, S or null
  MUTAGEN (10)..(10): Xaa is N, T, R, K or null
  MUTAGEN (11)..(11): Xaa is Y, F, S, N or null
  MUTAGEN (12)..(12): Xaa is Y or null
XXXXXXXXXXXX

SEQ ID NO: 5 - protein, 3 aa, Artificial Sequence
  LCDR2
  MUTAGEN (1)..(1): Xaa is T, K, G, W, E, M, L, D, A or Q
  MUTAGEN (2)..(2): Xaa is V, A, T or G
  MUTAGEN (3)..(3): Xaa is S or A
XXX

SEQ ID NO: 6 - protein, 13 aa, Artificial Sequence
  LCDR3
  MUTAGEN (1)..(1): Xaa is M, Q, L or H
  MUTAGEN (2)..(2): Xaa is G, Y, A, V, H, T, F or S
  MUTAGEN (3)..(3): Xaa is T, G, Y, N, L, D or S
  MUTAGEN (4)..(4): Xaa is H, S, T, Q, D, N, G, I or R
  MUTAGEN (5)..(5): Xaa is W, S, T, Y, L, I or N
  MUTAGEN (6)..(6): Xaa is P, S, M, I, W or
  MUTAGEN (7)..(7): Xaa is W, F, L, P, I, Y, R or T
  MUTAGEN (8)..(8): Xaa is T, L, A, F or W
  MUTAGEN (9)..(9): Xaa is F, L, T or null
  MUTAGEN (10)..(10): Xaa is T, F or null
  MUTAGEN (11)..(11): Xaa is F or null
  misc_feature (12)..(13): Xaa can be any naturally occurring amino acid
CXQXXXXXXXXXX

SEQ ID NO: 7 - protein, 9 aa, Artificial Sequence
  CDR
GASIINNNW

SEQ ID NO: 8 - protein, 9 aa, Artificial Sequence
  CDR
GDSISSSYW

SEQ ID NO: 9 - protein, 9 aa, Artificial Sequence
  CDR
GDSISSTNW

SEQ ID NO: 10 - protein, 10 aa, Artificial Sequence
  CDR
GFSLSTSAVN

SEQ ID NO: 11 - protein, 10 aa, Artificial Sequence
  CDR
GFSLSTSGVG

SEQ ID NO: 12 - protein, 8 aa, Artificial Sequence
  CDR
GFTFDDYA

SEQ ID NO: 13 - protein, 8 aa, Artificial Sequence
  CDR
GFTFSDYY

SEQ ID NO: 14 - protein, 8 aa, Artificial Sequence
  CDR
GFTFSNAW

SEQ ID NO: 15 - protein, 8 aa, Artificial Sequence
  CDR
GFTFSNYW

SEQ ID NO: 16 - protein, 9 aa, Artificial Sequence
  CDR
GGSINSSSW

SEQ ID NO: 17 - protein, 9 aa, Artificial Sequence
  CDR
GGSINSTNW

SEQ ID NO: 18 - protein, 9 aa, Artificial Sequence
  CDR
GGSISNGNW

SEQ ID NO: 19 - protein, 9 aa, Artificial Sequence
  CDR
GGSISNSNW

SEQ ID NO: 20 - protein, 9 aa, Artificial Sequence
  CDR
GGSISRSNW

SEQ ID NO: 21 - protein, 9 aa, Artificial Sequence
  CDR
GGSISSSIW

SEQ ID NO: 22 - protein, 9 aa, Artificial Sequence
  CDR
GGSISSSKW

SEQ ID NO: 23 - protein, 9 aa, Artificial Sequence
  CDR
GGSISSSNW

SEQ ID NO: 24 - protein, 9 aa, Artificial Sequence
  CDR
GGSISSTNW

SEQ ID NO: 25 - protein, 9 aa, Artificial Sequence
  CDR
GGSISSYNW

SEQ ID NO: 26 - protein, 9 aa, Artificial Sequence
  CDR
GVSISSSNW

SEQ ID NO: 27 - protein, 8 aa, Artificial Sequence
  CDR
GYIFTRYA

SEQ ID NO: 28 - protein, 8 aa, Artificial Sequence
  CDR
GYIFTSYA

SEQ ID NO: 29 - protein, 8 aa, Artificial Sequence
  CDR
GYTFANFG

SEQ ID NO: 30 - protein, 8 aa, Artificial Sequence
  CDR
GYTFIGYY

SEQ ID NO: 31 - protein, 8 aa, Artificial Sequence
  CDR
GYTFTGYF

SEQ ID NO: 32 - protein, 8 aa, Artificial Sequence
  CDR
GYTFTGYY

SEQ ID NO: 33 - protein, 8 aa, Artificial Sequence
  CDR
GYTFTNYA

SEQ ID NO: 34 - protein, 8 aa, Artificial Sequence
  CDR
GYTFTNYG

SEQ ID NO: 35 - protein, 8 aa, Artificial Sequence
  CDR
GYTFTRYT

SEQ ID NO: 36 - protein, 8 aa, Artificial Sequence
  CDR
GYTFTSYD

SEQ ID NO: 37 - protein, 8 aa, Artificial Sequence
  CDR
GYTFTSYG

SEQ ID NO: 38 - protein, 9 aa, Artificial Sequence
  CDR
SGSISSSIW

SEQ ID NO: 39 - protein, 8 aa, Artificial Sequence
  CDR
MNPNSGNT

SEQ ID NO: 40 - protein, 7 aa, Artificial Sequence
  CDR
IYWSDDK

SEQ ID NO: 41 - protein, 7 aa, Artificial Sequence
  CDR
IYQSGST

SEQ ID NO: 42 - protein, 7 aa, Artificial Sequence
  CDR
IYHSGST

SEQ ID NO: 43 - protein, 7 aa, Artificial Sequence
  CDR
IYHSGNT

SEQ ID NO: 44 - protein, 7 aa, Artificial Sequence
  CDR
IYHSGDT

SEQ ID NO: 45 - protein, 7 aa, Artificial Sequence
  CDR
IYHGGST

SEQ ID NO: 46 - protein, 8 aa, Artificial Sequence
  CDR
ISWNSGSI

SEQ ID NO: 47 - protein, 8 aa, Artificial Sequence
  CDR
ISSSGTTI

SEQ ID NO: 48 - protein, 7 aa, Artificial Sequence
  CDR
ISHNGST

SEQ ID NO: 49 - protein, 8 aa, Artificial Sequence
  CDR
ISGSDSTI

SEQ ID NO: 50 - protein, 8 aa, Artificial Sequence
  CDR
ISAYSGDK

SEQ ID NO: 51 - protein, 8 aa, Artificial Sequence
  CDR
ISAYNGYT

SEQ ID NO: 52 - protein, 8 aa, Artificial Sequence
  CDR
ISAYNGNT

SEQ ID NO: 53 - protein, 8 aa, Artificial Sequence
  CDR
ISAYNGHT

SEQ ID NO: 54 - protein, 8 aa, Artificial Sequence
  CDR
INPNSGGT

SEQ ID NO: 55 - protein, 8 aa, Artificial Sequence
  CDR
INPNSGAT

SEQ ID NO: 56 - protein, 8 aa, Artificial Sequence
  CDR
INPNNGDT

SEQ ID NO: 57 - protein, 7 aa, Artificial Sequence
  CDR
INHSGNT

SEQ ID NO: 58 - protein, 7 aa, Artificial Sequence
  CDR
INHNGST

SEQ ID NO: 59 - protein, 8 aa, Artificial Sequence
  CDR
INAGNGNT

SEQ ID NO: 60 - protein, 10 aa, Artificial Sequence
  CDR
IKSKADGGTI

SEQ ID NO: 61 - protein, 10 aa, Artificial Sequence
  CDR
IKRKTDGGTT

SEQ ID NO: 62 - protein, 8 aa, Artificial Sequence
  CDR
IKQDGSEK

SEQ ID NO: 63 - protein, 7 aa, Artificial Sequence
  CDR
IHHSGNT

SEQ ID NO: 64 - protein, 7 aa, Artificial Sequence
  CDR
IFWNDDK

SEQ ID NO: 65 - protein, 7 aa, Artificial Sequence
  CDR
IFHSGTT

SEQ ID NO: 66 - protein, 13 aa, Artificial Sequence
  CDR
CVRSGDWHCFDYW

SEQ ID NO: 67 - protein, 17 aa, Artificial Sequence
  CDR
CVKDYYGSGSYGDIQHW

SEQ ID NO: 68 - protein, 14 aa, Artificial Sequence
  CDR
CVIWFGELLSFDYW

SEQ ID NO: 69 - protein, 12 aa, Artificial Sequence
  CDR
CVGGGYDAFDIW

SEQ ID NO: 70 - protein, 15 aa, Artificial Sequence
  CDR
CVAYVSGTYYNFDYW

SEQ ID NO: 71 - protein, 16 aa, Artificial Sequence
  CDR
CTTDLYSSSWDAFDIW

SEQ ID NO: 72 - protein, 9 aa, Artificial Sequence
  CDR
CTSDYGDYW

SEQ ID NO: 73 - protein, 13 aa, Artificial Sequence
  CDR
CTSAARRGYFDIW

SEQ ID NO: 74 - protein, 11 aa, Artificial Sequence
  CDR
CTREAGPFDYW

SEQ ID NO: 75 - protein, 14 aa, Artificial Sequence
  CDR
CTHRPGYTYGYGYW

SEQ ID NO: 76 - protein, 13 aa, Artificial Sequence
  CDR
CSREGGNAFFDYW

SEQ ID NO: 77 - protein, 15 aa, Artificial Sequence
  CDR
CATLPGYSSGWFDSW

SEQ ID NO: 78 - protein, 12 aa, Artificial Sequence
  CDR
CASSGSLYMDVW

SEQ ID NO: 79 - protein, 9 aa, Artificial Sequence
  CDR
CASEDFDYW

SEQ ID NO: 80 - protein, 12 aa, Artificial Sequence
  CDR
CARYSTPFFDYW

SEQ ID NO: 81 - protein, 14 aa, Artificial Sequence
  CDR
CARVVVASYYFDNW

SEQ ID NO: 82 - protein, 12 aa, Artificial Sequence
  CDR
CARVGANWFDPW

SEQ ID NO: 83 - protein, 13 aa, Artificial Sequence
  CDR
CARTGPTVTTDYW

SEQ ID NO: 84 - protein, 13 aa, Artificial Sequence
  CDR
CARTGPIVTTEYW

SEQ ID NO: 85 - protein, 13 aa, Artificial Sequence
  CDR
CARSGTTHTFDIW

SEQ ID NO: 86 - protein, 19 aa, Artificial Sequence
  CDR
CARSGLYEWELQYYYMDVW

SEQ ID NO: 87 - protein, 15 aa, Artificial Sequence
  CDR
CARMGYYYGSGSDYW

SEQ ID NO: 88 - protein, 16 aa, Artificial Sequence
  CDR
CARKGYNWNYDYFDYW

SEQ ID NO: 89 - protein, 11 aa, Artificial Sequence
  CDR
CARGGTTFDYW

SEQ ID NO: 90 - protein, 18 aa, Artificial Sequence
  CDR
CARGGLYLYSSSWFFDSW

SEQ ID NO: 91 - protein, 12 aa, Artificial Sequence
  CDR
CARGGAVALDYW

SEQ ID NO: 92 - protein, 11 aa, Artificial Sequence
  CDR
CARGDVLLWFG

SEQ ID NO: 93 - protein, 11 aa, Artificial Sequence
  CDR
CARGDILLWFG

SEQ ID NO: 94 - protein, 17 aa, Artificial Sequence
  CDR
CAREWFGELWQIFFDYW

SEQ ID NO: 95 - protein, 14 aa, Artificial Sequence
  CDR
CAREGVGATPFDYW

SEQ ID NO: 96 - protein, 12 aa, Artificial Sequence [sequence omitted]

SEQ ID NO: 97 - protein, 16 aa, Artificial Sequence
  CDR
CARDWEGFGESIGDYW

SEQ ID NO: 98 - protein, 15 aa, Artificial Sequence
  CDR
CARDWAGDRYYFDYW

SEQ ID NO: 99 - protein, 15 aa, Artificial Sequence
  CDR
CARDWAGDHYYFDYW

SEQ ID NO: 100 - protein, 17 aa, Artificial Sequence
  CDR
CARDSSTWYEGNYFDYW

SEQ ID NO: 101 - protein, 19 aa, Artificial Sequence
  CDR
CARDRDVYGYSGYGYFDYW

SEQ ID NO: 102 - protein, 16 aa, Artificial Sequence
  CDR
CARDQDYYGSGNFYYW

SEQ ID NO: 103 - protein, 17 aa, Artificial Sequence
  CDR
CARDQADYFGSGNYVYW

SEQ ID NO: 104 - protein, 18 aa, Artificial Sequence
  CDR
CARDPYGSGTYYRLFDYW

SEQ ID NO: 105 - protein, 10 aa, Artificial Sequence
  CDR
CARDPPSDYW

SEQ ID NO: 106 - protein, 16 aa, Artificial Sequence
  CDR
CARDEDYYGSGNYYHW

SEQ ID NO: 107 - protein, 13 aa, Artificial Sequence
  CDR
CARAGTGTTLDYW

SEQ ID NO: 108 - protein, 13 aa, Artificial Sequence
  CDR
CAQYNWNSSFDYW

SEQ ID NO: 109 - protein, 9 aa, Artificial Sequence
  CDR
CANEDFDYW

SEQ ID NO: 110 - protein, 13 aa, Artificial Sequence
  CDR
CAKSGTYGYFDYW

SEQ ID NO: 111 - protein, 16 aa, Artificial Sequence
  CDR
CAKDKGIMVRGGPDYW

SEQ ID NO: 112 - protein, 10 aa, Artificial Sequence
  CDR
CAHYSNYDYW

SEQ ID NO: 113 - protein, 13 aa, Artificial Sequence
  CDR
CAGEDTGWPFDFW

SEQ ID NO: 114 - protein, 12 aa, Artificial Sequence
  CDR
CAETSTITTNYW

SEQ ID NO: 115 - protein, 6 aa, Artificial Sequence
  CDR
HGSSTY

SEQ ID NO: 116 - protein, 6 aa, Artificial Sequence
  CDR
QDINTY

SEQ ID NO: 117 - protein, 6 aa, Artificial Sequence
  CDR
QDISDY

SEQ ID NO: 118 - protein, 6 aa, Artificial Sequence
  CDR
QDISNY

SEQ ID NO: 119 - protein, 6 aa, Artificial Sequence
  CDR
QGIRND

SEQ ID NO: 120 - protein, 6 aa, Artificial Sequence
  CDR
QGIWND

SEQ ID NO: 121 - protein, 6 aa, Artificial Sequence
  CDR
QSISNW

SEQ ID NO: 122 - protein, 6 aa, Artificial Sequence
  CDR
QSISNY

SEQ ID NO: 123 - protein, 6 aa, Artificial Sequence
  CDR
QSISSW

SEQ ID NO: 124 - protein, 11 aa, Artificial Sequence
  CDR
QSLLHSNGYNY

SEQ ID NO: 125 - protein, 11 aa, Artificial Sequence
  CDR
QSLVYRDGNTF

SEQ ID NO: 126 - protein, 11 aa, Artificial Sequence
  CDR
QSLVYSDGDTY

SEQ ID NO: 127 - protein, 11 aa, Artificial Sequence
  CDR
QSLVYSDGHTS

SEQ ID NO: 128 - protein, 11 aa, Artificial Sequence
  CDR
QSLVYSDGNTF

SEQ ID NO: 129 - protein, 11 aa, Artificial Sequence
  CDR
QSLVYSDGNTN

SEQ ID NO: 130 - protein, 11 aa, Artificial Sequence
  CDR
QSLVYSDGNTY

SEQ ID NO: 131 - protein, 6 aa, Artificial Sequence
  CDR
QSTSSY

SEQ ID NO: 132 - protein, 12 aa, Artificial Sequence
  CDR
QSVFYSSNSRNY

SEQ ID NO: 133 - protein, 12 aa, Artificial Sequence
  CDR
QSVLYSSNNKNY

SEQ ID NO: 134 - protein, 7 aa, Artificial Sequence
  CDR
QSVSGDY

SEQ ID NO: 135 - protein, 7 aa, Artificial Sequence
  CDR
QSVSGNY

SEQ ID NO: 136 - protein, 7 aa, Artificial Sequence
  CDR
QSVSGSY

SEQ ID NO: 137 - protein, 7 aa, Artificial Sequence
  CDR
QSVSSGY

SEQ ID NO: 138 - protein, 6 aa, Artificial Sequence
  CDR
QSVSSN

SEQ ID NO: 139 - protein, 7 aa, Artificial Sequence
  CDR
QSVSSNY

SEQ ID NO: 140 - protein, 7 aa, Artificial Sequence
  CDR
QSVSSRY

SEQ ID NO: 141 - protein, 7 aa, Artificial Sequence
  CDR
QSVSSSY

SEQ ID NO: 142 - protein, 7 aa, Artificial Sequence
  CDR
QSVSSTY

SEQ ID NO: 143 - protein, 6 aa, Artificial Sequence
  CDR
QTISSY

SEQ ID NO: 144 - protein, 7 aa, Artificial Sequence
  CDR
QTVSGNY

SEQ ID NO: 145 - protein, 7 aa, Artificial Sequence
  CDR
QTVSSSY

SEQ ID NO: 146 - protein, 3 aa, Artificial Sequence
  CDR
TVS

SEQ ID NO: 147 - protein, 3 aa, Artificial Sequence
  CDR
KVS

SEQ ID NO: 148 - protein, 3 aa, Artificial Sequence
  CDR
GAS

SEQ ID NO: 149 - protein, 3 aa, Artificial Sequence
  CDR
WAS

SEQ ID NO: 150 - protein, 3 aa, Artificial Sequence
  CDR
EVS

SEQ ID NO: 151 - protein, 3 aa, Artificial Sequence
  CDR
MAS

SEQ ID NO: 152 - protein, 3 aa, Artificial Sequence
  CDR
GTS

SEQ ID NO: 153 - protein, 3 aa, Artificial Sequence
  CDR
LGS

SEQ ID NO: 154 - protein, 3 aa, Artificial Sequence
  CDR
DAS

SEQ ID NO: 155 - protein, 3 aa, Artificial Sequence
  CDR
AAS

SEQ ID NO: 156 - protein, 3 aa, Artificial Sequence
  CDR
WTS

SEQ ID NO: 157 - protein, 3 aa, Artificial Sequence
  CDR
DAF

SEQ ID NO: 158 - protein, 3 aa, Artificial Sequence
  CDR
QVS

SEQ ID NO: 159 - protein, 3 aa, Artificial Sequence
  CDR
KAA

SEQ ID NO: 160 - protein, 11 aa, Artificial Sequence [sequence omitted]

SEQ ID NO: 161 - protein, 11 aa, Artificial Sequence [sequence omitted]

SEQ ID NO: 162 - protein, 11 aa, Artificial Sequence [sequence omitted]

SEQ ID NO: 163 - protein, 11 aa, Artificial Sequence [sequence omitted]

SEQ ID NO: 164 - protein, 11 aa, Artificial Sequence [sequence omitted]

SEQ ID NO: 165 - protein, 11 aa, Artificial Sequence [sequence omitted]

SEQ ID NO: 166 - protein, 11 aa, Artificial Sequence [sequence omitted]

SEQ ID NO: 167 - protein, 11 aa, Artificial Sequence [sequence omitted]

SEQ ID NO: 168 - protein, 11 aa, Artificial Sequence [sequence omitted]

SEQ ID NO: 169 - protein, 11 aa, Artificial Sequence [sequence omitted]

SEQ ID NO: 170 - protein, 13 aa, Artificial Sequence
  CDR
CQQYGGSPPLLTF

SEQ ID NO: 171 - protein, 11 aa, Artificial Sequence [sequence omitted]

SEQ ID NO: 172 - protein, 11 aa, Artificial Sequence [sequence omitted]

SEQ ID NO: 173 - protein, 11 aa, Artificial Sequence
  CDR
CQQYGSSMFTF

SEQ ID NO: 174 - protein, 11 aa, Artificial Sequence [sequence omitted]

SEQ ID NO: 175 - protein, 11 aa, Artificial Sequence [sequence omitted]

SEQ ID NO: 176 - protein, 11 aa, Artificial Sequence [sequence omitted]

SEQ ID NO: 177 - protein, 11 aa, Artificial Sequence [sequence omitted]

SEQ ID NO: 178 - protein, 11 aa, Artificial Sequence [sequence omitted]

SEQ ID NO: 179 - protein, 11 aa, Artificial Sequence [sequence omitted]

SEQ ID NO: 180 - protein, 11 aa, Artificial Sequence [sequence omitted]

SEQ ID NO: 181 - protein, 11 aa, Artificial Sequence [sequence omitted]

SEQ ID NO: 182 - protein, 11 aa, Artificial Sequence [sequence omitted]

SEQ ID NO: 183 - protein, 11 aa, Artificial Sequence [sequence omitted]

SEQ ID NO: 184 - protein, 11 aa, Artificial Sequence [sequence omitted]

SEQ ID NO: 185 - protein, 11 aa, Artificial Sequence [sequence omitted]

SEQ ID NO: 186 - protein, 11 aa, Artificial Sequence [sequence omitted]

SEQ ID NO: 187 - protein, 11 aa, Artificial Sequence [sequence omitted]

SEQ ID NO: 188 - protein, 11 aa, Artificial Sequence [sequence omitted]

SEQ ID NO: 189 - protein, 11 aa, Artificial Sequence [sequence omitted]

SEQ ID NO: 190 - protein, 13 aa, Artificial Sequence [sequence omitted]

SEQ ID NO: 191 - protein, 11 aa, Artificial Sequence [sequence omitted]

SEQ ID NO: 192 - protein, 10 aa, Artificial Sequence [sequence omitted]

SEQ ID NO: 193 - protein, 11 aa, Artificial Sequence [sequence omitted]

SEQ ID NO: 194 - protein, 10 aa, Artificial Sequence
  CDR
CQQYYDYWTF

SEQ ID NO: 195 - protein, 11 aa, Artificial Sequence [sequence omitted]

SEQ ID NO: 196 - protein, 12 aa, Artificial Sequence [sequence omitted]

SEQ ID NO: 197 - protein, 11 aa, Artificial Sequence [sequence omitted]

SEQ ID NO: 198 - protein, 11 aa, Artificial Sequence [sequence omitted]

SEQ ID NO: 199 - protein, 11 aa, Artificial Sequence
  CDR
CQQYNNYTFTF

SEQ ID NO: 200 - protein, 114 aa, Artificial Sequence
  VH
QVQLQESGPGLVKPSGTLSLTCVVSGGSISSSNWWNWVRQSPGKGLEWIGEINHSGNTNYNPSLKSRVTISVDKSKNQFSLNLSTLTAADTAVYYCASEDFDYWGQGTLVTVSS

SEQ ID NO: 201 - protein, 112 aa, Artificial Sequence
  VH
DVVMTQSPLSLPVTLGQPASISCRSSQSLVYSDGDTYLNWFQQRPGQSPRRLIYTVSYRDSGVPDRFSGSGSGTDFTLKISRVEAEDVGVYFCMQGTHWPWTFGQGTKVEIK

SEQ ID NO: 202 - protein, 114 aa, Artificial Sequence
  VH
QVQLQESGPGLVKPSGTLSLSCAFSGGSISSSNWWNWVRQSPGKGLEWIGEINHSGNTSYNPSLKSRVTISVDRSKNQFSLKLSSVTAADTAVYYCASEDFDYWGQGTLVTVSS

SEQ ID NO: 203 - protein, 112 aa, Artificial Sequence; identical to SEQ ID NO: 201
  VH

SEQ ID NO: 204 - protein, 114 aa, Artificial Sequence
  VH
QVQLQESGPGLVKPSGTLSLTCAVSGGSISSSNWWNWVRQPPGKGLEWIGEIYHSGNTSFNPSLKSRVTISVDKSKNQLSLNLTSVTAADTAIYYCASEDFDYWGQGTLVTVSS

SEQ ID NO: 205 - protein, 112 aa, Artificial Sequence
  VH
DVVMTQSPLSLPVTLGQPASISCRSSQSLVYSDGDTYLNWFQQRPGQSPRRLIYKVSNRDSGVPDRFSGSGSGTDFTLKISRVEAEDVGVYYCMQGTHWPWTFGQGTKVEIK

SEQ ID NO: 206 - protein, 114 aa, Artificial Sequence
  VH
QVQLQESGPGLVKPSGTLSLTCAVSGGSISSSNWWNWVRQPPGKGLEWIGEISHNGSTNYNPSLKSRVTISVDKSKNQFSLKLSSVTAADTAVYYCASEDFDYWGQGTLVTVSS

SEQ ID NO: 207 - protein, 112 aa, Artificial Sequence
  VH
DVVMTQSPLSLPVTLGQPASISCRSSQSLVYSDGDTYLNWFQQRPGQSPRRLIYKVSNRDSGVPDRFSGSGSGTDFTLKISRVEAEDVGFYYCMQGTHWPWTFGQGTKVEIK

SEQ ID NO: 208 - protein, 120 aa, Artificial Sequence
  VH
QVQLVQSGAEVKKPGASVKVSCKASGYTFTNYGISWVRQAPGQGLEWMGWISAYSGDKKYEQKFQGRVSVTTDTSTSTVYMELRSLRSDDTAVYYCARDWAGDHYYFDYWGQGTLVTVSS

SEQ ID NO: 209 - protein, 108 aa, Artificial Sequence
  VH
EIVLTQSPGTLSLSPGERATLSCRASQSVSSSYLVWYQQKPGQAPRLLIYGASSRATGIPDRFSGSGSGTDFTLTISRLEPEDFAVYYCQQYGSSPFTFGPGTKVDIK

SEQ ID NO: 210 - protein, 118 aa, Artificial Sequence
  VH
QVQLVQSGAEVKKPGASVKISCKASGYTFTRYTIHWVRQAPGQRLEWMGWINAGNGNTKYSQKFQGRVTITRDTSASTAYMELSSLRSEDTAVYYCAKSGTYGYFDYWGQGTLVTVSS

SEQ ID NO: 211 - protein, 113 aa, Artificial Sequence
  VH
DIVMTQSPDSLAVSLGERATINCKSSQSVLYSSNNKNYLVWYQQKPGQPPKLLIYWASTRESGVPDRFSGSGSGTDFTLTISSLQAEDVAVYYCQQYYSTPLTFGGGTKVEIK

SEQ ID NO: 212 - protein, 117 aa, Artificial Sequence
  VH
QVQLVQSGAEVKKPGASVKVSCKASGYIFTRYAMHWVRQAPGQRLEWMGWINAGNGNTKYSQKFQDRVTITRDTSASTAYMELSSLRSEDTAVYYCVGGGYDAFDIWGQGTMVTVSS

SEQ ID NO: 213 - protein, 112 aa, Artificial Sequence
  VH
DVVMTQSPLSLPVTLGQPASISCRSSQSLVYSDGNTYLIWFQQRPGQSPRRLIYEVSNRDSGVPDRFSGSGSGTDFTLKISRVEAEDVGVYYCMQGTHWPPTFGQGTKVEIK

SEQ ID NO: 214 - protein, 117 aa, Artificial Sequence
  VH
QVQLVQSGAEVKKPGASVKVSCKASGYIFTSYAMHWVRQAPGQRLEWMGWINAGNGNTKYSQKFQGRVTITRDTSASTAYMELSSLRSEDTAVYYCVGGGYDAFDIWGQGTMVTVSS

SEQ ID NO: 215 - protein, 112 aa, Artificial Sequence
  VH
DVVMTQSPLSLPVTLGQPASISCRSSQSLVYRDGNTFLFWFQQRPGQSPRRLVYEVSNRDSGVPDRFSGSGSDTDFTLKISRVEAEDVGVYYCMQGTHWPPTFGQGTKVEIK

SEQ ID NO: 216 - protein, 115 aa, Artificial Sequence
  VH
QVPLVQSGAEVKKPGASVKVSCKASGYTFTGYYMHWVRQAPGQGLEWVGRINPNNGDTNYAQKFQGRVTMTRDTSISTAYMELSRLRSGDTAVYYCARDPPSDYWGQGTLVTVSS

SEQ ID NO: 217 - protein, 107 aa, Artificial Sequence
  VH
DIQMTQSPSTLSASVGDRVTITCRASQSISNWLAWYQQKPGRAPKLLIYMASSLETGVPSRFSGSGSGTEFTLTISSLQPDDFATYYCQQYNSYSLTFGGGTKVEIK

SEQ ID NO: 218 - protein, 118 aa, Artificial Sequence
  VH
QVQLQESGPGLVKPSGTLSLTCAVSGGSISSSNWWNWVRQPPGKGLEWIGEIYHSGSTNFNPSLKSRVSILVDKSKNQFSLKLSSVTAADTAVYYCARSGTTHTFDIWGQGTMVTVSS

SEQ ID NO: 219 - protein, 108 aa, Artificial Sequence
  VH
EIVLTQSPGTLSLSPGERATLSCRASQTVSGNYLAWYQQKPGQAPRLLIYGTSFRATGIPDNFSGSGSGTDFTLTISRLEPEDFAVYYCQQYGTSPITFGQGTRLEIK

SEQ ID NO: 220 - protein, 122 aa, Artificial Sequence
  VH
EVQLVESGGGLVQPGRSLRLSCAASGFTFDDYAMHWVRQAPGKGLEWVSGISWNSGSIYYVDSVKGRFTISRDNAKNSLYLQMNSLRAEDTALYYCVKDYYGSGSYGDIQHWGQGTLVTVSS

SEQ ID NO: 221 - protein, 112 aa, Artificial Sequence
  VH
DIVMTQSPLSLPVTPGEPASISCRSSQSLLHSNGYNYLDWYLQKPGQSPQLLIYLGSNRASGVPDRFSGSGSGTDFTLKIRRVEAEDVGVYYCMQALQTPYTFGQGTKLEIK

SEQ ID NO: 222 - protein, 123 aa, Artificial Sequence
  VH
EVQLVESGGGLVKPGGSLRLSCAASGFTFSNAWMTWVRQAPGKGLEWVGRIKSKADGGTIDYAAPVKGRFTLSRDDSRNTLYLQMNSLKPEDTAVYYCTTDLYSSSWDAFDIWGQGTMVTVSS

SEQ ID NO: 223 - protein, 107 aa, Artificial Sequence
  VH
DIQMTQSPSSLSASVGDRVTITCQASQDISDYLNWYQQKPGKAPKLLIYDASNLETGVPSRFSGSGSGTDFTFTISSLQPEDLATYYCQQYDDLPLTFGGGTKVEIR

SEQ ID NO: 224 - protein, 120 aa, Artificial Sequence
  VH
QVQLVQSGAEVKKPGASVKVSCKASGYTFTNYGISWVRQAPGQGLEWIGWISAYNGNTNYAQKLQGRVSVTTDTSTNTAYMELRSLRSDDTAVYYCARDWAGDRYYFDYWGQGTLVTVSS

SEQ ID NO: 225 - protein, 108 aa, Artificial Sequence
  VH
EIVLTQSPGTLSLSPGERATLSCRASQSVSSNYLVWYQQKPGQAPRLLIYGASSRATGIPDRFSGSGSGTDFTLTISRLEPEDFAVYYCQQYGSSPLTFGGGTKVEIK

SEQ ID NO: 226 - protein, 120 aa, Artificial Sequence
  VH
QITLKESGPTLVKPTQTLTLTCTFSGFSLSTSGVGVGWIRQPPGKALEWLALIYWSDDKRYSPSLKSRLTITKDTSKNQVVLTMTNMDPVDTATYYCTHRPGYTYGYGYWGQGTLVTVSS

SEQ ID NO: 227 - protein, 112 aa, Artificial Sequence
  VH
DVVMTQSPLSLPVTLGQPASISCRSSQSLVYSDGNTFLHWFQQRPGQSPRRLIYKVSNRDSGVPDRFSGSGSGTDFTLKISRVEAEDVGLYYCMQGTHWPWTFGQGTKVEIK

SEQ ID NO: 228 - protein, 114 aa, Artificial Sequence; identical to SEQ ID NO: 206
  VH

SEQ ID NO: 229 - protein, 107 aa, Artificial Sequence
  VH
DIQMTQSPSSLSASVGDRVTITCQASQDISNYLNWYQQKPGKAPKLLIYDASNLETGVPSRFSGSGSGTDFTFTISSLQPEDIATYYCQQYDNLPITFGQGTRLEIK

SEQ ID NO: 230 - protein, 118 aa, Artificial Sequence
  VH
QVQLQESGPGLVKPSGTLSLTCAVSGGSISSSIWWSWVRQPPGKGLEWIGEIHHSGNTNCNPSLKSRVTISIDKSKNQFSLKLTSVTAADTAVYYCARAGTGTTLDYWGQGTLVTVSS

SEQ ID NO: 231 - protein, 108 aa, Artificial Sequence
  VH
EIVLTQSPGTLSLSPGERATLSCRASQSVSGDYLAWYQQKLGQAPRLLIYGASIRATGIPDRFSGSGSGTDFTLTISKLEPEDFAVYYCQQYGSSPLTFGGGTKVEIK

SEQ ID NO: 232 - protein, 114 aa, Artificial Sequence; identical to SEQ ID NO: 200
  VH

SEQ ID NO: 233 - protein, 107 aa, Artificial Sequence; identical to SEQ ID NO: 223
  VH

SEQ ID NO: 234 - protein, 114 aa, Artificial Sequence
  VH
QVQLQESGPGLVKPSGTLSLTCAVSGGSISSSNWWNWVRQSPGKGLEWIGEINHSGNTNYNPSLKSRVTISIDKSKNQFSLKMSSVTAADTAMYYCANEDFDYWGQGTLVTVSS

SEQ ID NO: 235 - protein, 112 aa, Artificial Sequence
  VH
DVVMTQSPLSLPVTLGQPASISCRSSQSLVYSDGDTYLNWFQQRPGQSPRRLIYTVSNRDSGVPDRFSGSGSGTDFALKISRVEAEDVGVYFCMQGTHWPWTFGQGTKVEIK

SEQ ID NO: 236 - protein, 120 aa, Artificial Sequence; identical to SEQ ID NO: 208
  VH

SEQ ID NO: 237 - protein, 108 aa, Artificial Sequence
  VH
EIVLTQSPGTLSLSPGERATLSCRASQSVSSSYLVWYQQKPGQAPRLLIYGASSRATGIPDRFSGSGSGTDFTLTISRLEPEDFAVYYCQQYGSSPLTFGGGTKVEIK

SEQ ID NO: 238 - protein, 124 aa, Artificial Sequence
  VH
QVQLVQSGAEVKKPGASVKVSCKASGYTFTNYAMHWVRQAPGQRLEWMGWINAGNGNTKYSQKFQGRVTITRDTSASTAYMELSSLRSEDTAVFYCARSGLYEWELQYYYMDVWGIGTTVTVSS

SEQ ID NO: 239 - protein, 108 aa, Artificial Sequence
  VH
EIVLTQSPGTLSLSPGERATLSCRASQSVSGNYLAWYQQRPGQAPRLLIYGASYRATGVPDRFSGSGSGTDFTLTITRLESEDFAVYYCQQYGSSPLTFGGGTKVEIK

SEQ ID NO: 240 - protein, 118 aa, Artificial Sequence
  VH
QVQLQESGPGLVKPSGTLSLTCAVSSGSISSSIWWSWVRQPPGKGLEWIGEIYHSGNTNYNPSLKSRVTISVDKSKNQFSLRLSSVTAADTAVYFCARAGTGTTLDYWGQGTLVTVSS

SEQ ID NO: 241 - protein, 108 aa, Artificial Sequence; identical to SEQ ID NO: 239
  VH

SEQ ID NO: 242 - protein, 123 aa, Artificial Sequence
  VH
QVQLVQSGAEVKKPGASVKVSCKASGYTFTGYYMHWVRQAPGQGLEWMGRINPNSGGTNYAQKFQGRVTMTRDTSINTAYMDLSRLRSDDTAVYYCARGGLYLYSSSWFFDSWGQGTLVTVSS

SEQ ID NO: 243 - protein, 110 aa, Artificial Sequence
  VH
EIVLTQSPGTLSLSPGERATLSCRASQSVSSSYLAWYQQKPGQAPRLLIYGASSRATGIPDRFSGSGSGTDFTLTISRLEPEDFAVYYCQQYGGSPPLLTFGGGTKVEIK

SEQ ID NO: 244 - protein, 124 aa, Artificial Sequence; identical to SEQ ID NO: 238
  VH

SEQ ID NO: 245 - protein, 112 aa, Artificial Sequence
  VH
DIVMTQSPLSLPVTPGEPASISCRSSQSLLHSNGYNYLDWYLQKPGQSPQFLIYLGSNRASGVPDRFSGSGSGTDFTLKISRVEAEDVGVYYCMQVLQTPYTFGQGTKLEIK

SEQ ID NO: 246 - protein, 116 aa, Artificial Sequence
  VH
QVQLVQSGAEVKKPGASVKVSCKASGYTFTGYFLHWVRQAPGQGLEWMGRINPNSGATNYAQKFQGRVTVTRDTSISTAYMDLSRLRFDDTAVYYCTREAGPFDYWGQGTLVTVSS

SEQ ID NO: 247 - protein, 112 aa, Artificial Sequence
  VH
DVVMTQSPLSLPVTLGQPASISCRSSQSLVYSDGHTSLNWFQQRPGQSPRRLIYKVSNRDSGVPDRFSGSGSDTDFTLKISRLEAEDVGVYCCMQGTHWPRTFGQGTKVEIK

SEQ ID NO: 248 - protein, 123 aa, Artificial Sequence
  VH
QVQLQESGPGLVKPSGTLSLTCAVSGGSISSTNWWGWVRQPPGKGLEWIGEIYQSGSTYYNPSLKSRVTISVDKSKNQFSLKLSSVTAADTAVYYCARDPYGSGTYYRLFDYWGQGILVTVSS

SEQ ID NO: 249 - protein, 108 aa, Artificial Sequence
  VH
EIVLTQSPGTLSLSPGERATLSCRASQSVSSSYLAWYQQKPGQAPRLLIYGASSRATGIPDRFSGSGSGTDFTLTINRLEPEDFAVYYCQQYGSSMFTFGPGTNVDIK

SEQ ID NO: 250 - protein, 121 aa, Artificial Sequence
  VH
QVQLVQSGAEVKKPGASVKVSCKASGYTFTSYDINWVRQATGQGLEWMGWMNPNSGNTGYAQKFQGRVTMTRNTSISTAYMELSSLRSEDTAVYYCARKGYNWNYDYFDYWGQGTLVTVSS

SEQ ID NO: 251 - protein, 112 aa, Artificial Sequence
  VH
DIVMTQSPLSLPVTPGEPASISCRSSQSLLHSNGYNYLDWYLQKPGQSPQLLIYLGSNRASGVPDRFSGSGSGTDFTLKISRVEAEDVGVYYCMQALQTPLTFGGGTKVEIK

SEQ ID NO: 252 - protein, 115 aa, Artificial Sequence
  VH
QVQLVQSGAEVKKPGASVKVSCKASGYTFTGYYMHWVRQAPGQGLEWMGRINPNSGGTNYAQKFQGRVTMTRDTSISTAYMELSRLRSDDTAVYYCAHYSNYDYWGQGTLVTVSS

SEQ ID NO: 253 - protein, 107 aa, Artificial Sequence
  VH
DIQMTQSPSSLSASVGDRVTITCRASQGIRNDLGWYQQKPGKAPKRLIYAASSLQSGVPSRFSGSGSGTEFTLTISSLQPEDFATYYCLQHNSYPWTFGQGTKVEIK

SEQ ID NO: 254 - protein, 116 aa, Artificial Sequence; identical to SEQ ID NO: 246
  VH

SEQ ID NO: 255 - protein, 113 aa, Artificial Sequence
  VH
DIVMTQSPDSLAVSLGERATINCRSSQSVFYSSNSRNYLAWYQQKPGQPPKLLIYWASTRESGVPDRFSGSGSGTDFTLTLSSLQAEDVAVYYCQQYYSSPWTFGQGTKVEIK

SEQ ID NO: 256 - protein, 122 aa, Artificial Sequence
  VH
QVQLVHSGAEVKKPGASVKVSCKASGYTFIGYYIHWVRQAPGQGLEWMGRINPNSGGTNYTQKFQGRVTMTRDTSISTAYMELSRLRSDDTAVYYCAREWFGELWQIFFDYWGQGTLVTVSS

SEQ ID NO: 257 - protein, 107 aa, Artificial Sequence
  VH
EIVMTQSPATLSVSPGERATLSCRASQSVSSNLAWYQQKPGQAPRLLIFGASTRATGTPARFSGSGSGTEFILTISSLQSEDFAIYYCQQYNNWPLTFGGGTKVEIK

SEQ ID NO: 258 - protein, 121 aa, Artificial Sequence
  VH
EVQLVESGGGLVQPGRSLRLSCSASGFTFDDYAMHWVRQAPGKGLEWVSTISWNSGSIGYADSVKGRFTISRDNAKNSLYLQMNSLRAEDTALYYCAKDKGIMVRGGPDYWGQGTLVTVSS

SEQ ID NO: 259 - protein, 107 aa, Artificial Sequence
  VH
DIQMTQSPSSLSASVRDRVTITCQASQDISNYLNWYQQKPGKAPKLLIYDASNLETGVPSRFSGSGSGTDFTFTISSLQPEDIATYYCQQYDILPYTFGQGTKLEIK

SEQ ID NO: 260 - protein, 118 aa, Artificial Sequence
  VH
QVQLVQSGAEVKKPGASVKVSCKASGYTFTGYYMHWVRQAPGQGLEWMGRINPNSGGTNYAQKFQGRVTMTRDTSISTAYMELSRLRSDDTAVYYCSREGGNAFFDYWGQGTLVTVSS

SEQ ID NO: 261 - protein, 113 aa, Artificial Sequence
  VH
DIVMTQSPDSLAVSLGERATINCKSSQSVLYSSNNKNYLAWYQQKPGQPPKLLIYWTSTRESGVPDRFSGSGSGTDFTLTISSLQAEDMAVYYCQQYYSTPYTFGQGTQLEIK

SEQ ID NO: 262 - protein, 118 aa, Artificial Sequence
  VH
QVQLQESGPGLVKPSGTLSLTCAVSGGSISSSIWWSWVRQPPGKGLEWIGEIHHSGNTNCNPSLKSRVTISIDKSKNQFSLKLTYVTDADTAVYYCARAGTGTTLDYWGQGTLVTVSS

SEQ ID NO: 263 - protein, 108 aa, Artificial Sequence; identical to SEQ ID NO: 231
  VH

SEQ ID NO: 264 - protein, 118 aa, Artificial Sequence; identical to SEQ ID NO: 230
  VH

SEQ ID NO: 265 - protein, 108 aa, Artificial Sequence
  VH
EIVLTQSPGTLSLSPGERATLSCRASQSVSGDYLAWYQQKLGQAPRLLIYGASIRATGIPDRFSGSGSGTDFTLTISRLEPEDFAVYYCQQYGSSPLTFGGGTKVEIK

SEQ ID NO: 266 - protein, 118 aa, Artificial Sequence
  VH
QVQLQESGPGLVKPSGTLSLTCAVSGGSISSSIWWSWVRQPPGKGLEWIGEIYHSGNTNCNPSLKSRVTISIDKSKNQFSLKLTSVTAADTAVYYCARAGTGTTLDYWGQGTLVTVSS

SEQ ID NO: 267 - protein, 108 aa, Artificial Sequence; identical to SEQ ID NO: 231
  VH

SEQ ID NO: 268 - protein, 118 aa, Artificial Sequence
  VH
QVQLQESGPGLVKPSGTLSLTCAVSGGSISSSIWWSWVRQPPGKGLEWIGEIYHSGNTNCNPSLKSRVTISVDKSKNQFSLKLSSVTAADTAVYYCARAGTGTTLDYWGQGTLVTVSS

SEQ ID NO: 269 - protein, 108 aa, Artificial Sequence
  VH
EIVLTQSPGTLSLSPGERATLSCRASQSVSGDYLAWYQQKPGQAPRLLIYGASSRATGIPDRFSGSGSGTDFTLTISKLEPEDFAVYYCQQYGSSPLTFGGGTKVEIK

SEQ ID NO: 270 - protein, 118 aa, Artificial Sequence
  VH
QVQLQESGPGLVKPSGTLSLTCAVSSGSISSSIWWSWVRQPPGKGLEWIGEIYHSGNTNYNPSLKSRVTISVDKSKNQFSLRLSSVTAADTAVYYCARAGTGTTLDYWGQGTLVTVSS

SEQ ID NO: 271 - protein, 108 aa, Artificial Sequence
  VL
EIVLTQSPGTLSLSPGERATLSCRASQSVSGNYLAWYQQRPGQAPRLLIYGASYRATGVPDRFSGSGSGTDFTLTITRLEPEDFAVYYCQQYGSSPLTFGGGTKVEIK

SEQ ID NO: 272 - protein, 123 aa, Artificial Sequence; identical to SEQ ID NO: 222
  VL

SEQ ID NO: 273 - protein, 108 aa, Artificial Sequence; identical to SEQ ID NO: 219
  VL

SEQ ID NO: 274 - protein, 117 aa, Artificial Sequence
  VL
QVQLVQSGAEVKKPGASVKVSCKASGYTFTSYGISWVRQAPGQGLEWMGWISAYNGNTNYAQKLQGRVTMTTDTSTSTAYMELRSLRSDDTAVYYCARVGANWFDPWGQGTLVTVSS

SEQ ID NO: 275 - protein, 113 aa, Artificial Sequence
  VL
DIVMTQSPDSLAVSLGERATINCKSSQSVLYSSNNKNYLVWYQQTPGQPPKLLIYWASTRESGVPDRFSGSGSGTDFTLTISSLQAEDVAVYYCQQYYSIPLTFGGGTKVEIK

SEQ ID NO: 276 - protein, 114 aa, Artificial Sequence; identical to SEQ ID NO: 200
  VL

SEQ ID NO: 277 - protein, 108 aa, Artificial Sequence; identical to SEQ ID NO: 219
  VL

SEQ ID NO: 278 - protein, 118 aa, Artificial Sequence
  VL
QVQLQESGPGLVKPSGTLSLTCTVSGGSISNGNWWNWVRQPPGKGLEWIGEIYHSGNTNYNPSLKSRVTISVDRSKNQFSLNLSSVTAADTAVYYCVRSGDWHCFDYWGQGTLVTVSS

SEQ ID NO: 279 - protein, 108 aa, Artificial Sequence
  VL
EIVLTQSPGTLSLSPGERATLSCRASQSVSSSYLAWYQQKPGQAPRLLIYGASSRATGIPDRFSGSGSGTDFTLTISGLEPEDFVVYYCQQYGNSPLTFGPGTKVDIK

SEQ ID NO: 280 - protein, 116 aa, Artificial Sequence
  VL
QVQLQESGPGLVKPSGTLSLTCDVSGGSISSSNWWSWVRQPPGKGLEWIGEIYHSGSTNYNPSLKSRVTISVDKSKNQVSLKLNSVTAADTAVYYCARGDILLWFGGQGTLVTVSS

SEQ ID NO: 281 - protein, 108 aa, Artificial Sequence
  VL
EIVLTQSPGTLSLSPGERATLSCRASQSVSSRYLAWYQQKPGQAPRLLIYGASNRATGMPDRFSGSGSGTDFTLTISRLEPEDFAVYYCQQYGSSPITFGQGTRLEIK

SEQ ID NO: 282 - protein, 121 aa, Artificial Sequence
  VL
QVQLQESGPGLVKPSGTLSLTCAVSGGSISSYNWWSWVRQPPGKGLEWIGEIYHSGSTNYNPSLKSRVTISVDKSKNQFSLKLSSVTAADTAVYYCARDEDYYGSGNYYHWGQGTLVTVSS

SEQ ID NO: 283 - protein, 108 aa, Artificial Sequence
  VL
EIVLTQSPGTLSLSPGERATLSCRASQSVSSSYLAWYQQKPGQAPRLLIYGASSRATGIPDRFSGSGSGTDFTLTISRLEPEDFAVFYCQQYGSLPLTFGGGTKVETK

SEQ ID NO: 284 - protein, 121 aa, Artificial Sequence
  VL
QVQLQESGPGLVKPSGTLSLTCAVSGGSISSYNWWSWVRQPPGKGLEWIGEIYHSGNTNYNPSLKSRVTISVDKSKNQFSLKLSSVTAADTAMYYCARDQDYYGSGNFYYWGQGTLVTVSS

SEQ ID NO: 285 - protein, 108 aa, Artificial Sequence
  VL
EIVLTQSPGTLSLSPGERATLSCRASQSVSSSYLAWYQQKPGQAPRLLIYGASSRATGIPDRFSGSGSGTDFTLTISRLEPEDFAVYYCQQYGSSPLTFGGGTKVEIK

SEQ ID NO: 286 - protein, 116 aa, Artificial Sequence
  VL
QVQLQESGPGLVKPSGTLSLTCAVSGGSISSSNWWSWVRQPPGKGLEWIGEIYHSGSTTYNPSLKSRVTISVDKSKSQISLKLTSVTAADTAVYYCARGDVLLWFGGRGTLVTVSS

SEQ ID NO: 287 - protein, 108 aa, Artificial Sequence
  VL
EIVLTQSPGTLSLSPGERASLSCRASQSVSSNYLAWYQQKPGQTPRLLIYGASIRATGIPDRFSGSGSGTDFTLIISRLEPEDFAVYYCQQYSSSPITFGQGTRLEIK

SEQ ID NO: 288 - protein, 116 aa, Artificial Sequence
  VL
QVQMQESGPGLVKPSGTLSLTCAVSGGSISSSKWWSWVRQPPGKGLEWIGEIYHSGSTNYNPSLKSRVTISIDKSKNQFSLRLTSVTAADTAVYYCARGDVLLWFGGQGTLVTVSS

SEQ ID NO: 289 - protein, 108 aa, Artificial Sequence
  VL
EIVLTQSPGTLSLSPGERATLSCWASQSVSSTYLAWYQQKPGQAPRLLIYGASIRATGIPDRFSGSGSGTDFTLTISSLEPEDFAVYYCQQYGSSPITFGQGTRLEIK

SEQ ID NO: 290 - protein, 116 aa, Artificial Sequence
  VL
QVQLQESGPGLVKPSGTLSLTCAVSGGSISSSNWWSWVRQPPGKGLEWIGEIYHSGNTNYNPSLKSRVTISVDKSKNQFSLKLSSVTAADTAVYYCARGGTTFDYWGQGTLVTVSS

SEQ ID NO: 291 - protein, 108 aa, Artificial Sequence
  VL
EIVLMQYPGTLSLSSGERATLSCRASQSVSSRYLAWYQQKPGQAPRLLIYGASNRASGMPDRFSGSGSGTEFTLTISSLEPEDFAMYYCQQYGSSPITFGQGTRVEIK

SEQ ID NO: 292 - protein, 120 aa, Artificial Sequence
  VL
QVQLQESGPGLVKPSGTLSLTCAVSGGSISSSNWWSWVRQPPGKGLEWIGEIYHGGSTNYNPSLKSRITISVDKSKNQFSLKLSSVTAADTAMYYCATLPGYSSGWFDSWGQGTLVTVSS

SEQ ID NO: 293 - protein, 108 aa, Artificial Sequence
  VL
EIVLMQSPGTLSLSPGERATLSCRASQSVSSSYLAWYQQKPGQAPSLLIYGASNRASGIPDRFSGSGSGTDFTLTITRLEPEDFAVYYCQQYGSSPLTFGGGTRVEIK

SEQ ID NO: 294 - protein, 118 aa, Artificial Sequence
  VL
QVQLQESGPGLVKLSGTLSLTCAVCGGSISSSNWWSWVRQIPGKRAGVDWGNLSWEHQLQPAPQESSHHISRQVQEPVLPEAELCDRRGHDRVLLCENGVLLWFGELLGPGNPGHRLL

SEQ ID NO: 295 - protein, 108 aa, Artificial Sequence
  VL
EIVLTQSPGTLSLSPGERATFSCRASQSVSGSYLAWYQQKPGQAPRLLIYGASSRATGIPDRFSGSGSGTDFTLTISRLEPEDFAVYYCLQYGSSPLTFGRGTKVEIK

SEQ ID NO: 296 - protein, 118 aa, Artificial Sequence
  VL
QVQLQESGPGLVKPAGTLSLTCAVSGGSISSSNWWNWVRQPPGKGLEWIGEIYHSGSTNYNPSLKSRVTISVDTSKNQFSLKLTSVTAADTAVYYCARTGPTVTTDYWGQGTLVTVSS

SEQ ID NO: 297 - protein, 108 aa, Artificial Sequence
  VL
EIVLTQSPGTLSLSPGERATLSCRASQSVSSSYLAWYQQKPGQAPRLLIYGASYRATGMPERFSGSGSGTDFTLTISRLEPEDFAIYYCQQYGRSPLTFGGGTKVEIK

SEQ ID NO: 298 - protein, 117 aa, Artificial Sequence
  VL
QVQLQESGPGLVKPSGTLSLTCAVSGVSISSSNWWSWVRQPPGKGLEWIGEIYHSGNTNYNPSLKSRVTISVDKSKNQFSLKLSSVTAADTAVYYCAETSTITTNYWGQGTLVTVSS

SEQ ID NO: 299 - protein, 107 aa, Artificial Sequence
  VL
DIQMTQSPSSLSASVGDRVTITCRASQTISSYLNWYQQKPGKAPKLLIYAASSLQSGVPSRFSGSESGTDFTLTISSLQPEDFATYYCQQTYSIPITFGQGTRLEIK

SEQ ID NO: 300 - protein, 117 aa, Artificial Sequence
  VL
QVQLQESGPGLVKPSETLSLTCAVSGGSINSTNWWSWVRQPPGKGLEWIGEIYHSGSTNYNPSLKSRVTISVDKSKNQFSLKLSSVTAADTAVYYCARGGAVALDYWGQGTLVTVSS

SEQ ID NO: 301 - protein, 108 aa, Artificial Sequence
  VL
EIVLTQSPGPLSLSPGDRATLSCRASQTVSSSYLAWYLQKPGQAPRLLIYGASIRATGIPDRFSGSGSGTDFTLTISRLEPEDFAVYYCQQYGNSPITFGQGTRLEIK

SEQ ID NO: 302 - protein, 116 aa, Artificial Sequence; identical to SEQ ID NO: 280
  VL

SEQ ID NO: 303 - protein, 107 aa, Artificial Sequence
  VL
DIQMTQSPSSLSASVGDRVTITCQASQDISNYLNWYQQKPGKAPKLLIYDAFNLEVGVPSRFSGSGSGTDFTFTISSLQPEDIATYYCQQYDNLPFTFGPGTKVDIK

SEQ ID NO: 304 - protein, 114 aa, Artificial Sequence
  VL
QVQLVQSGAEVKKPGASVKVSCKASGYTFTSYGISWVRQAPGQGLEWMGWISAYNGHTNYAQKLQGRVTMTTDTSTNTAYMELWSLRSDDTAVYYCTSDYGDYWGQGTLVTVSS

SEQ ID NO: 305 - protein, 114 aa, Artificial Sequence
  VL
DVVVTQSPLSLPVTLGQPASISCRSSQSLVYSDGNTNLYWFQQRPGQSPRRLIYQVSNRDSGVPDRFSGSGSGTDFTLKISRVEAEDVGVYYCMQGTHWPPALTFGGGTEVEIK

SEQ ID NO: 306 - protein, 116 aa, Artificial Sequence
  VL
QVQMQESGPGLVKPSGTLSLICAVSGGSISSSKWWSWVRQPPGKGLEWIGEIYHSGSTNYNPSLKSRVTISIDKSKNQFSLRLTSVTAADTAVYYCARGDVLLWFGGQGTLVTVSS

SEQ ID NO: 307 - protein, 108 aa, Artificial Sequence; identical to SEQ ID NO: 283
  VL

SEQ ID NO: 308 - protein, 120 aa, Artificial Sequence
  VL
QVQLQESGPGLVKPSGNLSLTCVVSGASIINNNWWTWVRQSPGKGLEWIGEIFHSGTTNYNPSLKNRVTISVDKAKNQFSLNLKSVTAADTAVYYCVAYVSGTYYNFDYWGQGTLVTVSS

SEQ ID NO: 309 - protein, 108 aa, Artificial Sequence
  VL
EIVLTQSPGTLSLSPGERATLSCRASQSVSGSYLAWYQQKPGQAPRLLIYGASSRATGIPDRFSGSGSGTDFTLTISRLEPEDFAVYYCQQFGSSPLTFGGGTKVEIK

SEQ ID NO: 310 - protein, 119 aa, Artificial Sequence
  VL
QVQLVQSGAEVKKPGASVKVSCKASGYTFTGYYIHWVRQAPGQGLEWMGRINPNSGGTDFAQKFQARVTMTRDTAINIVYMELSRLRSDDTAVYYCARVVVASYYFDNWGQGTLVTVSS

SEQ ID NO: 311 - protein, 112 aa, Artificial Sequence; identical to SEQ ID NO: 251
  VL

SEQ ID NO: 312 - protein, 124 aa, Artificial Sequence
  VL
QVQLVESGGGLVKPGGSLRLSCAASGFTFSDYYMSWIRQAPGRGLEWISYISGSDSTIYYEDSVMGRFTISRDNAKNSLYLQMNSLRAEDTAVYYCARDRDVYGYSGYGYFDYWGQGTLVTVSS

SEQ ID NO: 313 - protein, 108 aa, Artificial Sequence; identical to SEQ ID NO: 281
  VL

SEQ ID NO: 314 - protein, 118 aa, Artificial Sequence
  VL
QVQLQESGPGLVKPSGTLSLTCAVSGGSISSSNWWTWVRQPPGKGLEWIGEIYHSGSTNYNPSLKSRVTISVDKSKNQFSLKLSSVTAADTAVYYCARTGPIVTTEYWGQGTLVTVSS

SEQ ID NO: 315 - protein, 108 aa, Artificial Sequence
  VL
EIVLTQSPGTLSLSPGERATLSCRASQSVSSGYLAWYQQKPGQAPRLLIYGASIRATGIPDRFSGSGSGTDFTLTISRLEPEDFALYYCQQYGSSPLTFGGGTKVEIK

SEQ ID NO: 316 - protein, 119 aa, Artificial Sequence
  VL
QITLKESGPTLVKPTQTLTLTCTFSGFSLSTSAVNVGWIRQPHGKALEWLALIFWNDDKRYSPSLKNRLTITKDTSKDQVVLTMSNMDPVDTATYYCAQYNWNSSFDYWGQGTLVTVSS

SEQ ID NO: 317 - protein, 106 aa, Artificial Sequence
  VL
DIQMTQSPSSLSASLGDRVTITCQASQDINTYLNWYQQKPGKAPKVLIYDASNLETGVPSRFSGSGSGTDFTFTISSLQPEDIATFYCQQYDNLITFGGGTKVEIK

SEQ ID NO: 318 - protein, 120 aa, Artificial Sequence
  VL
EVQLVESGGGLVKPGGSLRLSCAASGFTFSNAWMSWVRQAPGKGLEWVGRIKRKTDGGTTDYATPVKGRFTISRDASKNTLYLQMNSLKTEDTAVYYCTSAARRGYFDIWGRGTLVTVSS

SEQ ID NO: 319 - protein, 108 aa, Artificial Sequence
  VL
EIVLTQSPGTLSLSPGERATLSCRASQSVSSRYLAWYQQKPGQAPRLLIYGASNRATGMPDRFSGSGSGTDFTLTISRLEPEDFAMYYCQQYGSSPITFGQGTRLEIK

SEQ ID NO: 320 - protein, 117 aa, Artificial Sequence
  VL
QVQLQESGPGLVKPSGTLSLTCAVSGGSISRSNWWTWVRQSPGKGLEWIGEIYHSGNTNYNPSLKSRVTISLDKSKNQFSLKLSSVTAADTAVYYCASSGSLYMDVWGKGTTVTVSS

SEQ ID NO: 321 - protein, 107 aa, Artificial Sequence
  VL
DIQMTQSPSSLSASVGDRVTISCRASQSTSSYLNWYQQKPGKAPRLLIYGASSLQSGVPSRFSGSGSGTDFILTISSLQPEDFATYYCQQSYSIPITFGQGTRLEIK

SEQ ID NO: 322 - protein, 119 aa, Artificial Sequence
  VL
EVQLVESGGGLVQPGGSLRLSCAASGFTFSNYWMSWVRQAPGKGLEWVANIKQDGSEKYYVDSVKGRFTISRDNAKNSLYLQMNSLRAEDTAVYYCAREGVGATPFDYWGQGSLVTVSS

SEQ ID NO: 323 - protein, 106 aa, Artificial Sequence
  VL
DIQMTQSPSTLSASVGDRVTITCRASQSISSWLAWYQQKPGKAPKLLIYKAASLESGVPSRFSGSGSGTEFTLTIRSLQPDDFATYYCQQYYDYWTFGQGTKVEIK

SEQ ID NO: 324 - protein, 117 aa, Artificial Sequence
  VL
QVQLQESGPGLVKPSGTLSLTCAVSGDSISSTNWWSWVRQPPGKGLEWIGEINHNGSTYYNPSLKSRVTISVDKSKNQFSLKLRSVTAADTAVYYCAREDYYYMDVWGKGTTVTVSS

SEQ ID NO: 325 - protein, 107 aa, Artificial Sequence
  VL
DIQMTQSPSSLSASVGDRVTITCRTSQGIWNDLGWYQQKPGKAPKRLIYAASSLQSGVPSRFSGSESGTEFTLTISSLQPEDFATYYCLQYNNYPLTFGGGTKVEIK

SEQ ID NO: 326 - protein, 121 aa, Artificial Sequence; identical to SEQ ID NO: 282
  VL

SEQ ID NO: 327 - protein, 108 aa, Artificial Sequence
  VL
EIVMTQSPATLSVSPGERATLSCRASQSVSSNLAWYQQKPGQAPRLLIYGASIRATGIPARFSGSGSGTEFTLTISSLQSEDFAVYYCHQYNNWPPWTFGQGTKVEIK

SEQ ID NO: 328 - protein, 122 aa, Artificial Sequence
  VL
QVQLVESGGGLVKPGGSLRLSCAASGFTFSDYYMSWIRQAPGKGLEWVSYISSSGTTIYCADSVKGRFTISRDNAKNSLYLQMNSLRAEDTAVYYCARDSSTWYEGNYFDYWGQGTLVTVSS

SEQ ID NO: 329 - protein, 112 aa, Artificial Sequence
  VL
DVVVTQSPLSLPVTLGQPASISCRSSQSLVYSDGNTYLNWFQQRPGQSPRRLIYKVSNRDSGVPDRFSGSGSGTDFTLKISRVEAEDVGVYYCMQGTHWPRTFGQGTKVEIK

SEQ ID NO: 330 - protein, 122 aa, Artificial Sequence
  VL
QVQLQESGPGLVKPSGTLSLTCAVSGGSINSSSWWSWVRQPPGKGLEWIGEIYHSGDTNYNPSLKSRVAISVDKSKNQFSLKLSSVTAADTAVYYCARDQADYFGSGNYVYWGQGTLVTVSS

SEQ ID NO: 331 - protein, 108 aa, Artificial Sequence
  VL
EIVLMQYPGTLSLSSGERRVLSCRPSQSVSSSYLAWYQQKPGQAPRLLIYGASSRASGIPDRFSGSGSGTDFTLTISRLEPEDFAVYYCQQYGSLPITFGQGTRVEIK

SEQ ID NO: 332 - protein, 121 aa, Artificial Sequence
  VL
QVQLVQSGAEVKKPGASVKVSCKASGYTFTGYYMHWVRQAPGQGLEWMGRINPNSGGTNYAQKFQGRVTMARDTSISTAYMELSRLRSDDTAVYYCARDWEGFGESIGDYWGQGTLVTVSS

SEQ ID NO: 333 - protein, 108 aa, Artificial Sequence
  VL
EIVLTQSPGTLSLSPGERATFSCRASQSVSGSYLAWYQQKPGQAPRLLIHGASSRATGIPDRFSGSGSGTDFTLTISRLEPEDFAVYYCLQYGSSPLTFGGGTKVEIK

SEQ ID NO: 334 - protein, 117 aa, Artificial Sequence
  VL
QVQLQESGPGLVKPSGTLSLTCAVSGGSISNSNWWNWVRQPPGRGLEWIGEIYHSGSTNYNPSLKSRVTISVDKSKNQFSLKLTSVTAADTAVYYCARYSTPFFDYWGQGNLVTVSS

SEQ ID NO: 335 - protein, 107 aa, Artificial Sequence
  VL
DIQMTQSPSSLSASVGDRVTITCRASQSISNYLNWYQQKQGKAPKLLIYGASSLQSGVPSRFSGSGSGTDFTLTINSLQPEDFATYCCQQSYNNPLTFGGGTKVEIK

SEQ ID NO: 336 - protein, 117 aa, Artificial Sequence
  VL
QVQLQESGPGLVKPSGTLSLTCAVSGGSISSSNWWSWVRQPPGKGLEWIGEIYHSGNTIYNPSLKSRVTISLDKSKNQFSLKLSSVTAADTAVYYCASSGSLYMDVWGKGTTVTVSS

SEQ ID NO: 337 - protein, 107 aa, Artificial Sequence
  VL
DIQMTQSPSSLLSSVGDRVTISCRASHGSSTYLNWYQQKPGKAPRLLIYGASSLQSGVPSRFSGSGFGTDFILTISSMQPEDFATYYCQQSYSIPITFGQGTRLEIK

SEQ ID NO: 338 - protein, 119 aa, Artificial Sequence
  VL
QVQLVQSGAEVKKPGASMKVSCKASGYTFANFGINWVRQAPGQGLEWMGWISAYNGYTNYAQQFQGRITMTTDTSTSTAYMELRSLRSDDTAIYYCVIWFGELLSFDYWGQGTLVTVSS

SEQ ID NO: 339 - protein, 107 aa, Artificial Sequence
  VL
DIQMTQFPSSLSASVGDRVTITCRASQDISNYLAWFQQKPGKAPKSLIYAASSLQSGVPSKFSGNGFGTDFTFPLSRMQPEDFASSYCQQYNNYTFTFGRGTKVEIK

SEQ ID NO: 340 - protein, 118 aa, Artificial Sequence
  VL
QVQLQESGPGLVKPSGTLSLTCAVFGDSISSSYWWSWVRQPPGKGLEWIGEIYHSGSTHYNPSLKSRVTISVDKSKNHLSLKLISVTDADTAVYYCAGEDTGWPFDFWGQGTLVTVSS

SEQ ID NO: 341 - protein, 108 aa, Artificial Sequence
  VL
EIVLTQSPGTLSLSPGERATLSCRASQSVSSSYLAWYQQKPGQAPRLLIYGASSRATGIPDRFSGSGSGTDFTLTISRLEPEDFAVYYCQQYGSSPITFGQGTRLEIK

SEQ ID NO: 342 - protein, 336 aa, Artificial Sequence
  CH
AKTTPPSVYPLAPGCGDTTGSSVTLGCLVKGYFPESVTVTWNSGSLSSSVHTFPALLQSGLYTMSSSVTVPSSTWPSQTVTCSVAHPASSTTVDKKLEPSGPISTINPCPPCKECHKCPAPNLEGGPSVFIFPPNIKDVLMISLTPKVTCVVVDVSEDDPDVQISWFVNNVEVHTAQTQTHREDYNSTIRVVSTLPIQHQDWMSGKEFKCKVNNKDLPSPIERTISKIKGLVRAPQVYILPPPAEQLSRKDVSLTCLVVGFNPGDISVEWTSNGHTEENYKDTAPVLDSDGSYFIYSKLNMKTSKWEKTDSFSCNVRHEGLKNYYLKKTISRSPGK

SEQ ID NO: 343 - protein, 335 aa, Artificial Sequence
  CH
AKTTAPSVYPLAPVCGGTTGSSVTLGCLVKGYFPEPVTLTWNSGSLSSGVHTFPALLQSGLYTLSSSVTVTSNTWPSQTITCNVAHPASSTKVDKKIEPRVPITQNPCPPLKECPPCAAPDLLGGPSVFIFPPKIKDVLMISLSPMVTCVVVDVSEDDPDVQISWFVNNVEVHTAQTQTHREDYNSTLRVVSALPIQHQDWMSGKEFKCKVNNRALPSPIEKTISKPRGPVRAPQVYVLPPPAEEMTKKEFSLTCMITGFLPAEIAVDWTSNGRTEQNYKNTATVLDSDGSYFMYSKLRVQKSTWERGSLFACSVVHEVLHNHLTTKTISRSLGK

SEQ ID NO: 344 - protein, 324 aa, Artificial Sequence
  CH
AKTTPPSVYPLAPGSAAQTNSMVTLGCLVKGYFPEPVTVTWNSGSLSSGVHTFPAVLESDLYTLSSSVTVPSSPRPSETVTCNVAHPASSTKVDKKIVPRDCGCKPCICTVPEVSSVFIFPPKPKDVLTITLTPKVTCVVVDISKDDPEVQFSWFVDDVEVHTAQTQPREEQFNSTFRSVSELPIMHQDWLNGKEFKCRVNSAAFPAPIEKTISKTKGRPKAPQVYTIPPPKEQMAKDKVSLTCMITDFFPEDITVEWQWNGQPAENYKNTQPIMNTNGSYFVYSKLNVQKSNWEAGNTFTCSVLHEGLHNHHTEKSLSHSPGK

SEQ ID NO: 345 - protein, 326 aa, Artificial Sequence
  CH
ASTKGPSVFPLAPCSRSTSESTAALGCLVKDYFPEPVTVSWNSGALTSGVHTFPAVLQSSGLYSLSSVVTVPSSNFGTQTYTCNVDHKPSNTKVDKTVERKCCVECPPCPAPPVAGPSVFLFPPKPKDTLMISRTPEVTCVVVDVEHEDPEVQFNWYVDGVEVHNAKTKPREEQFNSTFRVVSVLTVVHQDWLNGKEYKCKVSNKGFPAPIEKTISKTKGQPREPQVYTLPPSREEMTKNQVSLTCLVKGFYPSDIAVEWESNGQPENNYKTTPPMLDSDGSFFLYSKLTVDKSRWQQGNVFSCSVMHEALHNHYTQKSLSLSPGK

SEQ ID NO: 346 - protein, 107 aa, Artificial Sequence
  CL
RADAAPTVSIFPPSSEQLTSGGASVVCFLNNFYPKDINVKWKIDGSERQNGVLNSWTDQDSKDSTYSMSSTLTLTKDEYERHNSYTCEATHKTSTSPIVKSFNRNEC

SEQ ID NO: 347 - protein, 107 aa, Artificial Sequence [sequence omitted]